European Patent Specification EP 3 880 304 B1, published October 16, 2024. Title: COMPOSITIONS FOR TREATING OXIDATIVE STRESS-ASSOCIATED SKIN DISEASES AND SKIN AGEING AND DIAGNOSIS OF OXIDATIVE STRESS-ASSOCIATED SKIN DISEASES. Applicant: S-Biomedic N.V. The sequence listing filed with the application follows.

SEQUENCE LISTING (21 sequences)

SEQ ID NO: 1 - protein, 161 aa, Cutibacterium acnes
MFVQIAASLAAASSIALGIPGAATPIDESQLPVGPQVSVTDSAQHTGPFAASSPLTITVKPGAPCVRADGYQESMVTRVLDDKGHQVWTGTFDESKLIGGTGLGTATFHVGSPAAAFNFHGSERTTYRTLSYCAYPHYVNGTRERLSQVSVKTFMVDPALN

SEQ ID NO: 2 - protein, 161 aa, Cutibacterium acnes
MFVQIAASLAAASSIALGIPGAATPIDESQLPVGPQVSVTDSAQHTGPFAASSPLTITVKPGAPCVRADGYQESMVTRVLDDKGHQVWTGTFDESKLIGGTGLGTATFHVGSPAAAFNFHGSERTTYRTLSYCAYPHYVNGTRERLSQVSVKTFMVDPTLN

SEQ ID NO: 3 - protein, 161 aa, Cutibacterium acnes
MFVQIAASLAAASSIALGMPGAATPIDESQLPVGPQVSVTDSAQHTGPFAASSPLAITVKPGAPCVRADGYQESMVTRVLDDKGHQVWTGTFDESKLIGGTGLGTATFHVESPAAAFNFHGNERTTYRTLSYCAYPHYVNGTRERLSQVSVKTFMVDPALN

SEQ ID NO: 4 - protein, 161 aa, Cutibacterium acnes
MFVQIAASLAAASTIALGVPGAATPLNGSQLPTGPQVSVTDPAQHTGPFSTATPLTIKVKPSAPCVRADGRQQSLVARVLDDKGHQVWSGTFDESQLIGGTGRGTATFHVGSAAAAFNFHGGKRTTYRALGYCAYPHYVNGTRERLSQVSVKTFTVDPAIN

SEQ ID NO: 5 - DNA, 142 bp, Cutibacterium acnes
aagccggaaggcagataaacctctacccgggacgccgtcgtctccaacaccttagtgacactatgcagtgctatgctccaaacgaaagtctaaatgattttcgctaatttccatacgtacgacatatcgggagaccatcatg

SEQ ID NO: 6 - DNA, 142 bp, Cutibacterium acnes; identical to SEQ ID NO: 5

SEQ ID NO: 7 - DNA, 143 bp, Cutibacterium acnes
aaaccgaaaggcaaacccaccccctaccgggcctaccgttgccgccggcacgtcgatgacactatgcagtgctacgctctagcagaaaattcatatgattttcgtcaattcccatacgtacgacatatcaggagatcgtcatg

SEQ ID NO: 8 - DNA, 143 bp, Cutibacterium acnes
aaaccgaaagacagacccaccccctaccggacataccgttgccgccaacacttcaatgacactatgcagtgctacgctctagtcgagaatctatatgattttcgtcaattcccatacgtacgacatatcgggagatcgtcatg

SEQ ID NO: 9 - DNA, 143 bp, Cutibacterium acnes
aaaccgaaaggcagacccaccccctaccgggcataccgttgccgccgacacttcgatgacactatgcagtgctatacttcagctgaaagtctatatgattttcgtcaattcccatacgtacgacatatcgggagatcgtcatg

SEQ ID NO: 10 - DNA, 143 bp, Cutibacterium acnes
aaaccgaaaggcagacccaccccctaccgggcataccgttgccgccgacacttcgatgacactatgcagtgctatacttcagctgaaaatctatatgattttcgtcaattcccatacgtacgacatatcgggagatcgtcatg

SEQ ID NO: 11 - DNA, 143 bp, Cutibacterium acnes
aaaccgaaaggcagacccaccccctaccgggcataccgttgccgccgacacttcgatgacactatgcagtgctacacttcaactgaaaatctatatgattttcgtcaattcccatacgtacgacatatcgggagatcgtcatg

SEQ ID NO: 12 - DNA, 143 bp, Cutibacterium acnes
aaaccgaaaggcagacccaccccctaccgggcataccgttgccgccgacacttcgatgacactatgcagtgctacacttcaactgaaaatctatatgattttcgtcaattcccatacgtacgacacatcgggagatcgtcatg

SEQ ID NO: 13 - DNA, 20 bp, Artificial sequence
  primer
gcatctagccctctcaccat

SEQ ID NO: 14 - DNA, 20 bp, Artificial sequence
  primer
ctgagagtccggtaggtggt

SEQ ID NO: 15 - DNA, 20 bp, Artificial sequence
  primer
gcatcatgactaccgtccac

SEQ ID NO: 16 - DNA, 20 bp, Artificial sequence
  primer
cggtggtctccttagaggtc

SEQ ID NO: 17 - DNA, 38 bp, Artificial sequence
  primer
ggctgaagctgaattcacacccatcgatgagagccaac

SEQ ID NO: 18 - DNA, 47 bp, Artificial sequence
  primer
gatgatgatggtcgactcctgctgcgccgttgagggcgggatccacc

SEQ ID NO: 19 - protein, 161 aa, Cutibacterium acnes; identical to SEQ ID NO: 4

SEQ ID NO: 20 - protein, 18 aa, Cutibacterium acnes
VRADGYQESMVTRVLDDK

SEQ ID NO: 21 - protein, 13 aa, Cutibacterium acnes
RTLSYCAYPHYVN